European Patent Application EP 4 435 109 A1, published September 25, 2024. Title: A promotor activation sequence, an expression vector containing the promotor activation sequence, and a mammal containing the expression vector. Applicant: Tokyo University of Pharmacy and Life Sciences. The sequence listing filed with the application follows.

SEQUENCE LISTING (18 sequences)

SEQ ID NO: 1 - DNA, 2549 bp, Homo sapiens
  source 1..2549: mol_type = unassigned DNA
ccaggaagttcaggaaattggctgacccagtgcatccatttggaagtgtagtgggcatctcgaaacgtaacatgcctgtgactgaagtcttgatttccttactcactctgaggcacctgccctcgggcaagagcatcaccatccgtccagtagcccagacagccgctgggtgtcatccttcacccccctttctttcccctttccctatatgaaatccatcaacaagtcctcccaccctccttctgaagccagtctcaaattcgtcccttcatcaacacctccaactgcctcctcgctggacttcctgctgccactctggctggccagtccattctccacccagcagccggggtgactttgcagatggaaatcatctcactcccccatggctttccaagatccagggcacccaggctcatctcctaggcctccaaagatggcgagatctggtctccgccccacattcagaccttgccccctcccctcactcctcttcccctccacctcttccatcatgacttctttctgtccctctgacaagccaacctggtttcaacctcaggacctttgtactagctgttccctccgtctgtgatgctcttcctccaggtcttcccgtggctcttcagtcttctggtcttctcagatcttcccttctcttgctgcccccacagtgcaggtattttatttttcttagcatttactattatgtggacttattttgttattgtatttggcttttttttttttttttaataagatagggagctcactattttgcccagactggtctcgaactcctacccacaagcgagtctgctttcacctgggcctcccaaagctctgggattactaggttgagcccccgcacctggcctgttaattgtatttgttgatgggtcagacgattattaggtgctcggcgaatgcttcttgaatgacttcaggtcatgagggatttcctgattctttcccggacaacacccgcaccgtccaaccgcccacttcccgaagcgaagagcccagtctggatgccaacctgttgacgtcttcccgcttggaagctgagcaggtgctcacaagcatggaggccacactcggaggccggatctgagtcactccctgcccgaggaacgctgcgttccggctgacgcgtcctcccgtaggccctggcgaggtcaacatccctgccacgcctcgcgctgcttgcggagctgcgcccaggggatgacctttttcctttgcgcggagaagggggcttgagaaacccgagctctgaaccaggtgggattcattcattcacgcatgcattcattcatgtagtcagtcagtcaatcagtcaacaaatatttgtcaaggccccacaatgtgctaggcactgttctaggtactgagggacacagcggtgcccgaggtagacaaggttcctgctcctcttgtgtttgtcatgcttgctggggagacggacaaggaaaatgataaagttaacagtaaatagtaaaggctgggccatggcgggagatgtgatcagagaaggcttctcagaggtcgtggccttgacagacgaacaggccaccgcacgcagtccctgctgaacctgcattcccagcgtctgtgtcaaagacccggggcggcaaaacgaccaggaggataaaagagcatcgcagtcgtaacggctgccgaaatagctcagttgggagagcgttagactgaagatctaaaggtccctggttcgatcccgggtttcggcacttcctctttttccttccccccgggggaaaaaggaggtgcatagacgaagccgattccttccaattgatcaaaggcttttactttctatatttaacaaagccccgagcagtgtccgcgaggagccagagggaaaggaaactccccctccactccccgtttgggtaaatcaaataaggtcaagtttttcccgtctccacctcctccatgtctcaaatgcacatttgttgatgcctgtttgttcatttttgctttctgttttttaacgtctgctttctgaactggaaacgatcgccttaaaatggcatgaagtcaagtcggacctgttgttttgtgggaaatacaagatacttaattctttggaaagtgtttagggaaagctacgtttaccttaaaacagtctcttgaagaacctgttttatgggcggtcctcgttagtatagtggtgagtatccccgcctgtcacgcgggagaccggggttcgattccccgacggggaggccaagtacgtttttaccattcttccgtatttttccttactcttcctatgaagaataaacccggcaggtaaacgggactctggttctgtggttgtctctggcctcgttgcgtgccacactgttacaggaaagcaagaaaaaggcagtgctcgcatgtggaagtgttcatccatttcgttctttttttttggagaccatttctttttttttttttttttcctcagacagagtctcgctctgtctcccaggctggagtgcagtggcccgatctcagctcactgtaacctccgccttccgggt

SEQ ID NO: 2 - DNA, 774 bp, Homo sapiens
  source 1..774: mol_type = unassigned DNA
cgcacgcagtccctgctgaacctgcattcccagcgtctgtgtcaaagacccggggcggcaaaacgaccaggaggataaaagagcatcgcagtcgtaacggctgccgaaatagctcagttgggagagcgttagactgaagatctaaaggtccctggttcgatcccgggtttcggcacttcctctttttccttccccccgggggaaaaaggaggtgcatagacgaagccgattccttccaattgatcaaaggcttttactttctatatttaacaaagccccgagcagtgtccgcgaggagccagagggaaaggaaactccccctccactccccgtttgggtaaatcaaataaggtcaagtttttcccgtctccacctcctccatgtctcaaatgcacatttgttgatgcctgtttgttcatttttgctttctgttttttaacgtctgctttctgaactggaaacgatcgccttaaaatggcatgaagtcaagtcggacctgttgttttgtgggaaatacaagatacttaattctttggaaagtgtttagggaaagctacgtttaccttaaaacagtctcttgaagaacctgttttatgggcggtcctcgttagtatagtggtgagtatccccgcctgtcacgcgggagaccggggttcgattccccgacggggaggccaagtacgtttttaccattcttccgtatttttccttactcttcctatgaagaataaacccggcaggtaaacgggactctggttctgtggttgtctctgg

SEQ ID NO: 3 - DNA, 29 bp, synthetic construct
  misc_feature 1..29: note = primer
  source 1..29: mol_type = other DNA
atccatggatcgactctagagggacagcc

SEQ ID NO: 4 - DNA, 41 bp, synthetic construct
  misc_feature 1..41: note = primer
  source 1..41: mol_type = other DNA
ataactagtcgacgcggccgcctcactgactccgtcctgga

SEQ ID NO: 5 - DNA, 29 bp, synthetic construct
  misc_feature 1..29: note = primer
  source 1..29: mol_type = other DNA
catgtcgacccagagacaaccacagaacc

SEQ ID NO: 6 - DNA, 29 bp, synthetic construct
  misc_feature 1..29: note = primer
  source 1..29: mol_type = other DNA
agtggtacccgcacgcagtccctgctgaa

SEQ ID NO: 7 - DNA, 29 bp, synthetic construct
  misc_feature 1..29: note = primer
  source 1..29: mol_type = other DNA
catgtcgacacccggaaggcggaggttac

SEQ ID NO: 8 - DNA, 29 bp, synthetic construct
  misc_feature 1..29: note = primer
  source 1..29: mol_type = other DNA
agtggtaccaggaagttcaggaaattggc

SEQ ID NO: 9 - DNA, 23 bp, synthetic construct
  misc_feature 1..23: note = primer
  source 1..23: mol_type = other DNA
ctagacccgggattggcgcgccg

SEQ ID NO: 10 - DNA, 23 bp, synthetic construct
  misc_feature 1..23: note = primer
  source 1..23: mol_type = other DNA
aattcggcgcgccaatcccgggt

SEQ ID NO: 11 - DNA, 35 bp, synthetic construct
  misc_feature 1..35: note = primer
  source 1..35: mol_type = other DNA
actggtaccatcgattcagccaggcacattagctc

SEQ ID NO: 12 - DNA, 29 bp, synthetic construct
  misc_feature 1..29: note = primer
  source 1..29: mol_type = other DNA
gaggtcgaccgggagcgggtgggcggccc

SEQ ID NO: 13 - DNA, 35 bp, synthetic construct
  misc_feature 1..35: note = primer
  source 1..35: mol_type = other DNA
tatgtcgacatcgatatacagacatgagctaatgt

SEQ ID NO: 14 - DNA, 29 bp, synthetic construct
  misc_feature 1..29: note = primer
  source 1..29: mol_type = other DNA
agtggtaccaggaagttcaggaaattggc

SEQ ID NO: 15 - DNA, 20 bp, synthetic construct
  misc_feature 1..20: note = Annealing sequence for production of multicloning site containingSalI site and KpnI site
  source 1..20: mol_type = other DNA
tcgagagtcggtaccatgcg

SEQ ID NO: 16 - DNA, 20 bp, synthetic construct
  misc_feature 1..20: note = Annealing sequence for production of multicloning site containingSalI site and KpnI site
  source 1..20: mol_type = other DNA
tcgacgcatggtaccgactc

SEQ ID NO: 17 - DNA, 78 bp, synthetic construct
  misc_feature 1..78: note = primer
  source 1..78: mol_type = other DNA
tagactagtaaattgtccgctaaattctggccgtttttggcttttttgttagacaatggtgagcaagggcgaggagga

SEQ ID NO: 18 - DNA, 43 bp, synthetic construct
  misc_feature 1..43: note = primer
  source 1..43: mol_type = other DNA
cttaggccggccactcgagtcagaagaactcgtcaagaaggcg